European Patent Application EP 4 141 017 A1, published March 1, 2023. Title: Duocarmycinderivative and use thereof. Applicant: Tohoku University. The sequence listing filed with the application follows.

SEQUENCE LISTING (13 sequences)

SEQ ID NO: 1 - protein, 133 aa, Artificial Sequence
  Description of Artificial Sequence: Recombinant protein
AEAGITGTWSDQLGDTFIVTAGADGALTGTYENAVGGAESRYVLTGRYDSAPATDGSGTALGWTVAWKNNSKNAHSATTWSGQYVGGADAKINTQWLLTSGTTNANAWKSTLVGHDTFTKVKPSAASHHHHHH

SEQ ID NO: 2 - protein, 241 aa, Artificial Sequence
  Description of Artificial Sequence: Recombinant protein
QVKLEQSGAEVVKPGASVKLSCKASGFNIKDSYMHWLRQGPGQRLEWIGWIDPENGDTEYAPKFQGKATFTTDTSANTAYLGLSSLRPEDTAVYYCNEGTPTGPYYFDYWGQGTLVTVSSGGGGSGGGGSGGGGSENVLTQSPSSMSVSVGDRVNIACSASSSVPYMHWLQQKPGKSPKLLIYLTSNLASGVPSRFSGSGSGTDYSLTISSVQPEDAATYYCQQRSSYPLTFGGGTKLEIK

SEQ ID NO: 3 - protein, 383 aa, Artificial Sequence
  Description of Artificial Sequence: Recombinant protein
QVKLEQSGAEVVKPGASVKLSCKASGFNIKDSYMHWLRQGPGQRLEWIGWIDPENGDTEYAPKFQGKATFTTDTSANTAYLGLSSLRPEDTAVYYCNEGTPTGPYYFDYWGQGTLVTVSSGGGGSGGGGSGGGGSENVLTQSPSSMSVSVGDRVNIACSASSSVPYMHWLQQKPGKSPKLLIYLTSNLASGVPSRFSGSGSGTDYSLTISSVQPEDAATYYCQQRSSYPLTFGGGTKLEIKGGGGSGGGGAEAGITGTWSDQLGDTFIVTAGADGALTGTYENAVGGAESRYVLTGRYDSAPATDGSGTALGWTVAWKNNSKNAHSATTWSGQYVGGADAKINTQWLLTSGTTNANAWKSTLVGHDTFTKVKPSAASHHHHHH

SEQ ID NO: 4 - protein, 405 aa, Artificial Sequence
  Description of Artificial Sequence: Recombinant protein
MKYLLPTAAAGLLLLAAQPAMAQVKLEQSGAEVVKPGASVKLSCKASGFNIKDSYMHWLRQGPGQRLEWIGWIDPENGDTEYAPKFQGKATFTTDTSANTAYLGLSSLRPEDTAVYYCNEGTPTGPYYFDYWGQGTLVTVSSGGGGSGGGGSGGGGSENVLTQSPSSMSVSVGDRVNIACSASSSVPYMHWLQQKPGKSPKLLIYLTSNLASGVPSRFSGSGSGTDYSLTISSVQPEDAATYYCQQRSSYPLTFGGGTKLEIKGGGGSGGGGAEAGITGTWSDQLGDTFIVTAGADGALTGTYENAVGGAESRYVLTGRYDSAPATDGSGTALGWTVAWKNNSKNAHSATTWSGQYVGGADAKINTQWLLTSGTTNANAWKSTLVGHDTFTKVKPSAASHHHHHH

SEQ ID NO: 5 - DNA, 1218 bp, Artificial Sequence
  Description of Artificial Sequence: Recombinant DNA
atgaaatatctgctgccgaccgcagcagcgggtctgctgctgctggcagcacagcctgcaatggcacaggttaaactggaacagagcggtgccgaagttgttaaaccgggtgcaagcgttaaactgagctgtaaagcaagcggctttaacatcaaagatagctatatgcattggctgcgtcagggtccgggtcagcgtctggaatggattggttggattgatccggaaaatggtgataccgaatatgcaccgaaatttcagggtaaagcaacctttaccaccgataccagcgcaaataccgcatatctgggtctgagcagcctgcgtccggaagataccgcagtgtattattgtaatgaaggcaccccgaccggtccgtattatttcgattattggggtcagggcaccctggttaccgttagcagcggtggtggtggtagtggtggcggtggttcaggcggtggcggtagcgaaaatgttctgacccagagcccgagcagcatgagcgttagcgttggtgatcgtgttaatattgcatgtagcgcaagcagcagcgttccgtacatgcactggctgcagcagaaaccgggtaaaagcccgaaactgctgatttatctgaccagcaatctggcaagcggtgttccgagccgttttagcggtagcggtagtggcaccgattatagcctgaccattagcagcgtgcagcctgaagatgcagcaacctattattgtcagcagcgtagcagttatccgctgacctttggtggtggcaccaaactggaaattaaagggggtggtggctcaggtggcggaggtgcagaagcaggtattaccggtacatggtcagatcagctgggtgatacctttattgttaccgcaggcgcagatggtgcactgaccggcacctatgaaaatgcagttggtggtgcagaaagccgttatgtgctgaccggtcgttatgatagcgcaccggcaaccgatggtagcggcaccgcactgggttggaccgttgcatggaaaaataacagcaaaaatgcacatagcgcaaccacctggtcaggtcagtatgtgggtggtgccgatgccaaaattaacacccagtggctgctgaccagcggtacaaccaatgcaaatgcctggaaaagtaccctggttggtcatgatacattcaccaaagttaaaccgagcgcagcaagccatcatcatcaccatcattaa

SEQ ID NO: 6 - protein, 141 aa, Artificial Sequence
  Description of Artificial Sequence: Recombinant protein
MDKIAIVNMGSLFQQVAQKTGVSNTLENEFKGRASELQRMETDLQAKMKKLQSMKAGSDRTKLEKDVMAQRQTFAQKAQAFEQDRARRSNEERGKLVTRIQTAVKSVANSQDIDLVVDANAVAYNSSDVKDITADVLKQVK

SEQ ID NO: 7 - protein, 9 aa, Artificial Sequence
  Description of Artificial Sequence: Recombinant linker
GGGGSGGGG

SEQ ID NO: 8 - DNA, 40 bp, Artificial Sequence
  Description of Artificial Sequence: Synthesized DNA
aaggagatatacatatggataaaattgccattgttaatat

SEQ ID NO: 9 - DNA, 39 bp, Artificial Sequence
  Description of Artificial Sequence: Recombinant protein
ttgagatctgccatatgttatttcacttgtttcagaacg

SEQ ID NO: 10 - DNA, 35 bp, Artificial Sequence
  Description of Artificial Sequence: Recombinant protein
agaaggagatataccatgaaatatctgctgccgac

SEQ ID NO: 11 - DNA, 36 bp, Artificial Sequence
  Description of Artificial Sequence: Recombinant protein
cgccgagctcgaattttaatgatggtgatgatgatg

SEQ ID NO: 12 - DNA, 26 bp, Artificial Sequence
  Description of Artificial Sequence: Recombinant protein
ggtatatctccttcttaaagttaaac

SEQ ID NO: 13 - DNA, 24 bp, Artificial Sequence
  Description of Artificial Sequence: Recombinant protein
aattcgagctcggcgcgcctgcag